European Patent Specification EP 3 684 412 B1, published February 14, 2024. Title: METHODS OF PREVENTING METHIONINE OXIDATION IN IMMUNOCONJUGATES. Applicant: IMMUNOGEN, INC. The sequence listing filed with the application follows.

SEQUENCE LISTING (23 sequences)

SEQ ID NO: 1 - protein, 11 aa, Artificial Sequence
  huCD123-6 LC-CDR1
RASQDINSYLS

SEQ ID NO: 2 - protein, 7 aa, Artificial Sequence
  huCD123-6 LC-CDR2
RVNRLVD

SEQ ID NO: 3 - protein, 9 aa, Artificial Sequence
  huCD123-6 LC-CDR3
LQYDAFPYT

SEQ ID NO: 4 - protein, 5 aa, Artificial Sequence
  huCD123-6 HC-CDR1
SSIMH

SEQ ID NO: 5 - protein, 17 aa, Artificial Sequence
  huCD123-6 HC-CDR2
YIKPYNDGTKYNEKFKG

SEQ ID NO: 6 - protein, 12 aa, Artificial Sequence
  huCD123-6 HC-CDR3
EGGNDYYDTMDY

SEQ ID NO: 7 - protein, 121 aa, Artificial Sequence
  huCD123-6Gv7 Heavy Chain Variable Region
QVQLVQSGAEVKKPGASVKVSCKASGYIFTSSIMHWVRQAPGQGLEWIGYIKPYNDGTKYNEKFKGRATLTSDRSTSTAYMELSSLRSEDTAVYYCAREGGNDYYDTMDYWGQGTLVTVSS

SEQ ID NO: 8 - protein, 450 aa, Artificial Sequence
  huCD123-6Gv7-C442 Heavy Chain Full Length
QVQLVQSGAEVKKPGASVKVSCKASGYIFTSSIMHWVRQAPGQGLEWIGYIKPYNDGTKYNEKFKGRATLTSDRSTSTAYMELSSLRSEDTAVYYCAREGGNDYYDTMDYWGQGTLVTVSSASTKGPSVFPLAPSSKSTSGGTAALGCLVKDYFPEPVTVSWNSGALTSGVHTFPAVLQSSGLYSLSSVVTVPSSSLGTQTYICNVNHKPSNTKVDKKVEPKSCDKTHTCPPCPAPELLGGPSVFLFPPKPKDTLMISRTPEVTCVVVDVSHEDPEVKFNWYVDGVEVHNAKTKPREEQYNSTYRVVSVLTVLHQDWLNGKEYKCKVSNKALPAPIEKTISKAKGQPREPQVYTLPPSRDELTKNQVSLTCLVKGFYPSDIAVEWESNGQPENNYKTTPPVLDSDGSFFLYSKLTVDKSRWQQGNVFSCSVMHEALHNHYTQKSLCLSPG

SEQ ID NO: 9 - protein, 108 aa, Artificial Sequence
  huCD123-6Gv4 Light Chain Variable Region
DIQMTQSPSSLSASVGDRVTITCRASQDINSYLSWFQQKPGKAPKTLIYRVNRLVDGVPSRFSGSGSGNDYTLTISSLQPEDFATYYCLQYDAFPYTFGQGTKVEIKR

SEQ ID NO: 10 - protein, 214 aa, Artificial Sequence
  huCD123-6Gv4 Light Chain Full Length
DIQMTQSPSSLSASVGDRVTITCRASQDINSYLSWFQQKPGKAPKTLIYRVNRLVDGVPSRFSGSGSGNDYTLTISSLQPEDFATYYCLQYDAFPYTFGQGTKVEIKRTVAAPSVFIFPPSDEQLKSGTASVVCLLNNFYPREAKVQWKVDNALQSGNSQESVTEQDSKDSTYSLSSTLTLSKADYEKHKVYACEVTHQGLSSPVTKSFNRGEC

SEQ ID NO: 11 - protein, 17 aa, Artificial Sequence
  huMy9-6 LC-CDR1
KSSQSVFFSSSQKNYLA

SEQ ID NO: 12 - protein, 7 aa, Artificial Sequence
  huMy9-6 LC-CDR2
WASTRES

SEQ ID NO: 13 - protein, 8 aa, Artificial Sequence
  huMy9-6 LC-CDR3
HQYLSSRT

SEQ ID NO: 14 - protein, 5 aa, Artificial Sequence
  huMy9-6 HC-CDR1
SYYIH

SEQ ID NO: 15 - protein, 17 aa, Artificial Sequence
  huMy9-6 HC-CDR2
VIYPGNDDISYNQKFQG

SEQ ID NO: 16 - protein, 9 aa, Artificial Sequence
  huMy9-6 HC-CDR3
EVRLRYFDV

SEQ ID NO: 17 - protein, 118 aa, Artificial Sequence
  huMy9-6 Heavy Chain Variable Region
QVQLQQPGAEVVKPGASVKMSCKASGYTFTSYYIHWIKQTPGQGLEWVGVIYPGNDDISYNQKFQGKATLTADKSSTTAYMQLSSLTSEDSAVYYCAREVRLRYFDVWGQGTTVTVSS

SEQ ID NO: 18 - protein, 447 aa, Artificial Sequence
  huMy9-6 Heavy Chain Full Length
QVQLQQPGAEVVKPGASVKMSCKASGYTFTSYYIHWIKQTPGQGLEWVGVIYPGNDDISYNQKFQGKATLTADKSSTTAYMQLSSLTSEDSAVYYCAREVRLRYFDVWGQGTTVTVSSASTKGPSVFPLAPSSKSTSGGTAALGCLVKDYFPEPVTVSWNSGALTSGVHTFPAVLQSSGLYSLSSVVTVPSSSLGTQTYICNVNHKPSNTKVDKKVEPKSCDKTHTCPPCPAPELLGGPSVFLFPPKPKDTLMISRTPEVTCVVVDVSHEDPEVKFNWYVDGVEVHNAKTKPREEQYNSTYRVVSVLTVLHQDWLNGKEYKCKVSNKALPAPIEKTISKAKGQPREPQVYTLPPSRDELTKNQVSLTCLVKGFYPSDIAVEWESNGQPENNYKTTPPVLDSDGSFFLYSKLTVDKSRWQQGNVFSCSVMHEALHNHYTQKSLSLSPG

SEQ ID NO: 19 - protein, 113 aa, Artificial Sequence
  huMy9-6 Light Chain Variable Region
EIVLTQSPGSLAVSPGERVTMSCKSSQSVFFSSSQKNYLAWYQQIPGQSPRLLIYWASTRESGVPDRFTGSGSGTDFTLTISSVQPEDLAIYYCHQYLSSRTFGQGTKLEIKR

SEQ ID NO: 20 - protein, 219 aa, Artificial Sequence
  huMy9-6 Light Chain Full Length
EIVLTQSPGSLAVSPGERVTMSCKSSQSVFFSSSQKNYLAWYQQIPGQSPRLLIYWASTRESGVPDRFTGSGSGTDFTLTISSVQPEDLAIYYCHQYLSSRTFGQGTKLEIKRTVAAPSVFIFPPSDEQLKSGTASVVCLLNNFYPREAKVQWKVDNALQSGNSQESVTEQDSKDSTYSLSSTLTLSKADYEKHKVYACEVTHQGLSSPVTKSFNRGEC

SEQ ID NO: 21 - protein, 4 aa, Artificial Sequence
  An embodiment of P in the immunoconjugate of formula (IA)
ALAL

SEQ ID NO: 22 - protein, 4 aa, Artificial Sequence
  An embodiment of P in the immunoconjugate of formula (IA), first Ala is beta-Ala
ALAL

SEQ ID NO: 23 - protein, 4 aa, Artificial Sequence
  An embodiment of P in the immunoconjugate of formula (IA)
GFLG